European Patent Application EP 4 122 956 A1, published January 25, 2023. Title: HIGH-AFFINITY TCR FOR RECOGNIZING AFP ANTIGEN. Applicant: XLIFESC, LTD. Application EP21770767.8. The sequence listing filed with the application follows.

SEQUENCE LISTING (68 sequences)

SEQ ID NO: 1 - protein, 111 aa, Artificial sequence
  synthesized polypeptide
GQNIDQPTEMTATEGAIVQINCTYQTSGFNGLFWYQQHAGEAPTFLSYNVLDGLEEKGRFSSFLSRSKGYSYLLLKELQMKDSASYLCAVRHFSDGQKLLFARGTMLKVDL

SEQ ID NO: 2 - protein, 114 aa, Artificial sequence
  synthesized polypeptide
KAGVTQTPRYLIKTRGQQVTLSCSPISGHRSVSWYQQTPGQGLQFLFEYFSETQRNKGNFPGRFSGRQFSNSRSEMNVSTLELGDSALYLCASSLGQGGKDEQYFGPGTRLTVT

SEQ ID NO: 3 - protein, 111 aa, Artificial sequence
  synthesized polypeptide
GQNIDQPTELTVTEGENVQINCTYQTSGFNGLFWYQQHAGEAPTFLSYNVLDGLEEKGRFSSFLSRSKGYSYLLIKEVQPKDSASYFCAVRHFSDGQKLLFARGTKLKVDP

SEQ ID NO: 4 - protein, 114 aa, Artificial sequence
  synthesized polypeptide
KAGVTQTPRYLSVTRGQQVTLSCSPISGHRSVSWYQQTPGQGLQFLFEYFSETQRNKGNFPGRFSGRQFSNSRSEMNISTVEPGDSALYFCASSLGQGGKDEQYFGPGTRLTVT

SEQ ID NO: 5 - DNA, 333 bp, Artificial sequence
  synthesized polynucleotide
ggtcaaaatattgatcaaccgaccgaactgaccgttaccgaaggtgaaaatgtgcagattaattgcacctatcagaccagcggttttaatggtctgttttggtatcagcagcatgcaggtgaagccccgacctttctgagctataatgttctggatggtctggaagaaaaaggtcgttttagtagctttctgagccgtagtaaaggttatagctatctgctgattaaggaagttcagccgaaagatagtgcaagctatttttgcgccgttcgtcattttagtgatggtcagaaactgctgtttgcccgcggcaccaaactgaaagttgatccg

SEQ ID NO: 6 - DNA, 342 bp, Artificial sequence
  synthesized polynucleotide
aaagcaggcgttacccagaccccgcgctatctgagtgttacccgcggccagcaggtgaccctgagctgtagtccgattagtggtcatcgcagtgtgagttggtatcagcaaaccccgggtcagggtctgcagtttctgtttgaatattttagtgaaacccagcgcaataagggcaattttccgggtcgtttttcaggtcgccagtttagtaatagccgtagcgaaatgaatattagcaccgtggaaccgggtgacagcgccctgtatttttgtgccagtagtctgggtcagggcggcaaagatgaacagtattttggcccgggcacccgtctgaccgtgacc

SEQ ID NO: 7 - protein, 24 aa, Artificial sequence
  synthesized polypeptide
GGGSEGGGSEGGGSEGGGSEGGTG

SEQ ID NO: 8 - DNA, 72 bp, Artificial sequence
  synthesized polynucleotide
ggtggtggcagtgaaggtggtggtagcgaaggtggtggctcagaaggtggtggaagtgaaggcggtaccggc

SEQ ID NO: 9 - protein, 249 aa, Artificial sequence
  synthesized polypeptide
GQNIDQPTELTVTEGENVQINCTYQTSGFNGLFWYQQHAGEAPTFLSYNVLDGLEEKGRFSSFLSRSKGYSYLLIKEVQPKDSASYFCAVRHFSDGQKLLFARGTKLKVDPGGGSEGGGSEGGGSEGGGSEGGTGKAGVTQTPRYLSVTRGQQVTLSCSPISGHRSVSWYQQTPGQGLQFLFEYFSETQRNKGNFPGRFSGRQFSNSRSEMNISTVEPGDSALYFCASSLGQGGKDEQYFGPGTRLTVT

SEQ ID NO: 10 - DNA, 747 bp, Artificial sequence
  synthesized polynucleotide
ggtcaaaatattgatcaaccgaccgaactgaccgttaccgaaggtgaaaatgtgcagattaattgcacctatcagaccagcggttttaatggtctgttttggtatcagcagcatgcaggtgaagccccgacctttctgagctataatgttctggatggtctggaagaaaaaggtcgttttagtagctttctgagccgtagtaaaggttatagctatctgctgattaaggaagttcagccgaaagatagtgcaagctatttttgcgccgttcgtcattttagtgatggtcagaaactgctgtttgcccgcggcaccaaactgaaagttgatccgggtggtggcagtgaaggtggtggtagcgaaggtggtggctcagaaggtggtggaagtgaaggcggtaccggcaaagcaggcgttacccagaccccgcgctatctgagtgttacccgcggccagcaggtgaccctgagctgtagtccgattagtggtcatcgcagtgtgagttggtatcagcaaaccccgggtcagggtctgcagtttctgtttgaatattttagtgaaacccagcgcaataagggcaattttccgggtcgtttttcaggtcgccagtttagtaatagccgtagcgaaatgaatattagcaccgtggaaccgggtgacagcgccctgtatttttgtgccagtagtctgggtcagggcggcaaagatgaacagtattttggcccgggcacccgtctgaccgtgacc

SEQ ID NO: 11 - protein, 206 aa, Artificial sequence
  synthesized polypeptide
MGQNIDQPTEMTATEGAIVQINCTYQTSGFNGLFWYQQHAGEAPTFLSYNVLDGLEEKGRFSSFLSRSKGYSYLLLKELQMKDSASYLCAVRHFSDGQKLLFARGTMLKVDLNIQNPDPAVYQLRDSKSSDKSVCLFTDFDSQTNVSQSKDSDVYITDKTVLDMRSMDFKSNSAVAWSNKSDFACANAFNNSIIPEDTFFCSPESS

SEQ ID NO: 12 - protein, 245 aa, Artificial sequence
  synthesized polypeptide
MKAGVTQTPRYLIKTRGQQVTLSCSPISGHRSVSWYQQTPGQGLQFLFEYFSETQRNKGNFPGRFSGRQFSNSRSEMNVSTLELGDSALYLCASSLGQGGKDEQYFGPGTRLTVTEDLKNVFPPEVAVFEPSECEISHTQKATLVCLATGFYPDHVELSWWVNGKEVHSGVSTDPQPLKEQPALNDSRYALSSRLRVSATFWQNPRNHFRCQVQFYGLSENDEWTQDRAKPVTQIVSAEAWGRAD

SEQ ID NO: 13 - protein, 111 aa, Artificial sequence
  synthesized polypeptide
GQNIDQPTEMTATEGAIVQINCTYQTSGFNGLFWYQQHAGEAPTFLSYNVLDGLEEKGRFSSFLSRSKGYSYLLLKELQMKDSASYLCAVRGWSDGQKLLFARGTMLKVDL

SEQ ID NO: 14 - protein, 111 aa, Artificial sequence
  synthesized polypeptide
GQNIDQPTEMTATEGAIVQINCTYQTSGFNGLFWYQQHAGEAPTFLSYNVLDGLEEKGRFSSFLSRSKGYSYLLLKELQMKDSASYLCAVRGWYDGQKLLFARGTMLKVDL

SEQ ID NO: 15 - protein, 111 aa, Artificial sequence
  synthesized polypeptide
GQNIDQPTEMTATEGAIVQINCTYQTSGFNGLFWYQQHAGEAPTFLSYNVLDGLEEKGRFSSFLSRSKGYSYLLLKELQMKDSASYLCAVRGWQDGQKLLFARGTMLKVDL

SEQ ID NO: 16 - protein, 111 aa, Artificial sequence
  synthesized polypeptide
GQNIDQPTEMTATEGAIVQINCTYQTSGFNGLFWYQQHAGEAPTFLSYNVLDGLEEKGRFSSFLSRSKGYSYLLLKELQMKDSASYLCAVRGWKDGQKLLFARGTMLKVDL

SEQ ID NO: 17 - protein, 111 aa, Artificial sequence
  synthesized polypeptide
GQNIDQPTEMTATEGAIVQINCTYQTSGFNGLFWYQQHAGEAPTFLSYNVLDGLEEKGRFSSFLSRSKGYSYLLLKELQMKDSASYLCAVRHWDGGQKLLFARGTMLKVDL

SEQ ID NO: 18 - protein, 111 aa, Artificial sequence
  synthesized polypeptide
GQNIDQPTEMTATEGAIVQINCTYQTSGFNGLFWYQQHAGEAPTFLSYNVLDGLEEKGRFSSFLSRSKGYSYLLLKELQMKDSASYLCAVRGWADGQKLLFARGTMLKVDL

SEQ ID NO: 19 - protein, 111 aa, Artificial sequence
  synthesized polypeptide
GQNIDQPTEMTATEGAIVQINCTYQTSGFNGLFWYQQHAGEAPTFLSYNVLDGLEEKGRFSSFLSRSKGYSYLLLKELQMKDSASYLCAVRGWHDGQKLLFARGTMLKVDL

SEQ ID NO: 20 - protein, 111 aa, Artificial sequence
  synthesized polypeptide
GQNIDQPTEMTATEGAIVQINCTYQTSGFNGLFWYQQHAGEAPTFLSYNVLDGLEEKGRFSSFLSRSKGYSYLLLKELQMKDSASYLCAVRGWIDGQKLLFARGTMLKVDL

SEQ ID NO: 21 - protein, 111 aa, Artificial sequence
  synthesized polypeptide
GQNIDQPTEMTATEGAIVQINCTYQTSGFNGLFWYQQHAGEAPTFLSYNVLDGLEEKGRFSSFLSRSKGYSYLLLKELQMKDSASYLCAVRGWLDGQKLLFARGTMLKVDL

SEQ ID NO: 22 - protein, 111 aa, Artificial sequence
  synthesized polypeptide
GQNIDQPTEMTATEGAIVQINCTYQTSGFNGLFWYQQHAGEAPTFLSYNVLDGLEEKGRFSSFLSRSKGYSYLLLKELQMKDSASYLCAVRGWMDGQKLLFARGTMLKVDL

SEQ ID NO: 23 - protein, 111 aa, Artificial sequence
  synthesized polypeptide
GQNIDQPTEMTATEGAIVQINCTYQTSGFNGLFWYQQHAGEAPTFLSYNVLDGLEEKGRFSSFLSRSKGYSYLLLKELQMKDSASYLCAVRGWNDGQKLLFARGTMLKVDL

SEQ ID NO: 24 - protein, 111 aa, Artificial sequence
  synthesized polypeptide
GQNIDQPTEMTATEGAIVQINCTYQTSGFNGLFWYQQHAGEAPTFLSYNVLDGLEEKGRFSSFLSRSKGYSYLLLKELQMKDSASYLCAVRGWRDGQKLLFARGTMLKVDL

SEQ ID NO: 25 - protein, 111 aa, Artificial sequence
  synthesized polypeptide
GQNIDQPTEMTATEGAIVQINCTYQTSGFNGLFWYQQHAGEAPTFLSYNVLDGLEEKGRFSSFLSRSKGYSYLLLKELQMKDSASYLCAVRGWTDGQKLLFARGTMLKVDL

SEQ ID NO: 26 - protein, 111 aa, Artificial sequence
  synthesized polypeptide
GQNIDQPTEMTATEGAIVQINCTYQTSGFNGLFWYQQHAGEAPTFLSYNVLDGLEEKGRFSSFLSRSKGYSYLLLKELQMKDSASYLCAVRHWNNGQKLLFARGTMLKVDL

SEQ ID NO: 27 - protein, 111 aa, Artificial sequence
  synthesized polypeptide
GQNIDQPTEMTATEGAIVQINCTYQTSGFNGLFWYQQHAGEAPTFLSYNVLDGLEEKGRFSSFLSRSKGYSYLLLKELQMKDSASYLCAVRHWQDGQKLLFARGTMLKVDL

SEQ ID NO: 28 - protein, 111 aa, Artificial sequence
  synthesized polypeptide
GQNIDQPTEMTATEGAIVQINCTYQTSGFNGLFWYQQHAGEAPTFLSYNVLDGLEEKGRFSSFLSRSKGYSYLLLKELQMKDSASYLCAVRHWSDGQKLLFARGTMLKVDL

SEQ ID NO: 29 - protein, 111 aa, Artificial sequence
  synthesized polypeptide
GQNIDQPTEMTATEGAIVQINCTYQTSGFNGLFWYQQHAGEAPTFLSYNVLDGLEEKGRFSSFLSRSKGYSYLLLKELQMKDSASYLCAVRHWQRGQKLLFARGTMLKVDL

SEQ ID NO: 30 - protein, 114 aa, Artificial sequence
  synthesized polypeptide
KAGVTQTPRYLIKTRGQQVTLSCSPISGHRSVSWYQQTPGQGLQFLFEYFSETQRNKGNFPGRFSGRQFSNSRSEMNVSTLELGDSALYLCASSLGQGGRMQEYFGPGTRLTVT

SEQ ID NO: 31 - protein, 114 aa, Artificial sequence
  synthesized polypeptide
KAGVTQTPRYLIKTRGQQVTLSCSPISGHRSVSWYQQTPGQGLQFLFEYFSETQRNKGNFPGRFSGRQFSNSRSEMNVSTLELGDSALYLCASASGVGGKDEQYFGPGTRLTVT

SEQ ID NO: 32 - protein, 114 aa, Artificial sequence
  synthesized polypeptide
KAGVTQTPRYLIKTRGQQVTLSCSPISGHRSVSWYQQTPGQGLQFLFEYFSETQRNKGNFPGRFSGRQFSNSRSEMNVSTLELGDSALYLCASSLGQGGRGTLYFGPGTRLTVT

SEQ ID NO: 33 - protein, 114 aa, Artificial sequence
  synthesized polypeptide
KAGVTQTPRYLIKTRGQQVTLSCSPISGHRSVSWYQQTPGQGLQFLFEYFSETQRNKGNFPGRFSGRQFSNSRSEMNVSTLELGDSALYLCASSLGQGGRDIQYFGPGTRLTVT

SEQ ID NO: 34 - protein, 205 aa, Artificial sequence
  synthesized polypeptide
GQNIDQPTEMTATEGAIVQINCTYQTSGFNGLFWYQQHAGEAPTFLSYNVLDGLEEKGRFSSFLSRSKGYSYLLLKELQMKDSASYLCAVRHFSDGQKLLFARGTMLKVDLNIQNPDPAVYQLRDSKSSDKSVCLFTDFDSQTNVSQSKDSDVYITDKTVLDMRSMDFKSNSAVAWSNKSDFACANAFNNSIIPEDTFFPSPESS

SEQ ID NO: 35 - protein, 244 aa, Artificial sequence
  synthesized polypeptide
KAGVTQTPRYLIKTRGQQVTLSCSPISGHRSVSWYQQTPGQGLQFLFEYFSETQRNKGNFPGRFSGRQFSNSRSEMNVSTLELGDSALYLCASSLGQGGKDEQYFGPGTRLTVTEDLKNVFPPEVAVFEPSEAEISHTQKATLVCLATGFYPDHVELSWWVNGKEVHSGVSTDPQPLKEQPALNDSRYCLSSRLRVSATFWQNPRNHFRCQVQFYGLSENDEWTQDRAKPVTQIVSAEAWGRAD

SEQ ID NO: 36 - protein, 252 aa, Artificial sequence
  synthesized polypeptide
GQNIDQPTEMTATEGAIVQINCTYQTSGFNGLFWYQQHAGEAPTFLSYNVLDGLEEKGRFSSFLSRSKGYSYLLLKELQMKDSASYLCAVRHFSDGQKLLFARGTMLKVDLNIQNPDPAVYQLRDSKSSDKSVCLFTDFDSQTNVSQSKDSDVYITDKTVLDMRSMDFKSNSAVAWSNKSDFACANAFNNSIIPEDTFFPSPESSCDVKLVEKSFETDTNLNFQNLSVIGFRILLLKVAGFNLLMTLRLWSS

SEQ ID NO: 37 - protein, 293 aa, Artificial sequence
  synthesized polypeptide
KAGVTQTPRYLIKTRGQQVTLSCSPISGHRSVSWYQQTPGQGLQFLFEYFSETQRNKGNFPGRFSGRQFSNSRSEMNVSTLELGDSALYLCASSLGQGGKDEQYFGPGTRLTVTEDLKNVFPPEVAVFEPSEAEISHTQKATLVCLATGFYPDHVELSWWVNGKEVHSGVSTDPQPLKEQPALNDSRYCLSSRLRVSATFWQNPRNHFRCQVQFYGLSENDEWTQDRAKPVTQIVSAEAWGRADCGFTSESYQQGVLSATILYEILLGKATLYAVLVSALVLMAMVKRKDSRG

SEQ ID NO: 38 - protein, 10 aa, Artificial sequence
  synthesized polypeptide
KWVESIFLIF

SEQ ID NO: 39 - protein, 6 aa, Artificial sequence
  synthesized polypeptide
TSGFNG

SEQ ID NO: 40 - protein, 6 aa, Artificial sequence
  synthesized polypeptide
NVLDGL

SEQ ID NO: 41 - protein, 12 aa, Artificial sequence
  synthesized polypeptide
AVRHFSDGQKLL

SEQ ID NO: 42 - protein, 5 aa, Artificial sequence
  synthesized polypeptide
SGHRS

SEQ ID NO: 43 - protein, 6 aa, Artificial sequence
  synthesized polypeptide
YFSETQ

SEQ ID NO: 44 - protein, 13 aa, Artificial sequence
  synthesized polypeptide
ASSLGQGGKDEQY

SEQ ID NO: 45 - protein, 12 aa, Artificial sequence
  synthesized polypeptide
AVRGWSDGQKLL

SEQ ID NO: 46 - protein, 12 aa, Artificial sequence
  synthesized polypeptide
AVRGWYDGQKLL

SEQ ID NO: 47 - protein, 12 aa, Artificial sequence
  synthesized polypeptide
AVRGWQDGQKLL

SEQ ID NO: 48 - protein, 13 aa, Artificial sequence
  synthesized polypeptide
ASSLGQGGRMQEY

SEQ ID NO: 49 - protein, 12 aa, Artificial sequence
  synthesized polypeptide
  variant (4)..(4): Xaa can be His or Gly
  variant (5)..(5): Xaa can be Phe or Trp
  variant (6)..(6): Xaa can be Gly, Tyr, Gln, Lys, Asp, Ala, His, Ile, Leu, Met, Asn, Arg or Thr
  variant (7)..(7): Xaa can be Asp, Arg, Gly or Asn
AVRXXXXGQKLL

SEQ ID NO: 50 - protein, 13 aa, Artificial sequence
  synthesized polypeptide
  variant (3)..(3): Xaa can be Ser or Ala
  variant (4)..(4): Xaa can be Ser or Leu
  variant (6)..(6): Xaa can be Gln or Val
  variant (9)..(9): Xaa can be Lys or Arg
  variant (10)..(10): Xaa can be Asp, Met or Gly
  variant (11)..(11): Xaa can be Glu, Gln or Thr
  variant (12)..(12): Xaa can be Gln, Glu or Leu
ASXXGXGGXXXXY

SEQ ID NO: 51 - protein, 12 aa, Artificial sequence
  synthesized polypeptide
AVRGWKDGQKLL

SEQ ID NO: 52 - protein, 12 aa, Artificial sequence
  synthesized polypeptide
AVRHWDGGQKLL

SEQ ID NO: 53 - protein, 12 aa, Artificial sequence
  synthesized polypeptide
AVRGWADGQKLL

SEQ ID NO: 54 - protein, 12 aa, Artificial sequence
  synthesized polypeptide
AVRGWHDGQKLL

SEQ ID NO: 55 - protein, 12 aa, Artificial sequence
  synthesized polypeptide
AVRGWIDGQKLL

SEQ ID NO: 56 - protein, 12 aa, Artificial sequence
  synthesized polypeptide
AVRGWLDGQKLL

SEQ ID NO: 57 - protein, 12 aa, Artificial sequence
  synthesized polypeptide
AVRGWMDGQKLL

SEQ ID NO: 58 - protein, 12 aa, Artificial sequence
  synthesized polypeptide
AVRGWNDGQKLL

SEQ ID NO: 59 - protein, 12 aa, Artificial sequence
  synthesized polypeptide
AVRGWRDGQKLL

SEQ ID NO: 60 - protein, 12 aa, Artificial sequence
  synthesized polypeptide
AVRGWTDGQKLL

SEQ ID NO: 61 - protein, 12 aa, Artificial sequence
  synthesized polypeptide
AVRHWNNGQKLL

SEQ ID NO: 62 - protein, 12 aa, Artificial sequence
  synthesized polypeptide
AVRHWQDGQKLL

SEQ ID NO: 63 - protein, 12 aa, Artificial sequence
  synthesized polypeptide
AVRHWSDGQKLL

SEQ ID NO: 64 - protein, 12 aa, Artificial sequence
  synthesized polypeptide
AVRHWQRGQKLL

SEQ ID NO: 65 - protein, 13 aa, Artificial sequence
  synthesized polypeptide
ASASGVGGKDEQY

SEQ ID NO: 66 - protein, 13 aa, Artificial sequence
  synthesized polypeptide
ASSLGQGGRGTLY

SEQ ID NO: 67 - protein, 13 aa, Artificial sequence
  synthesized polypeptide
ASSLGQGGRDIQY

SEQ ID NO: 68 - protein, 5 aa, Artificial sequence
  linker
GGGGS